European Patent Application EP 4 227 416 A1, published August 16, 2023. Title: HOMOGENEOUS BETA-1,3-GLUCAN/NUCLEIC ACID COMPLEXES, AND USE THEREOF. Applicant: NapaJen Pharma, Inc. The University of Kitakyushu. The sequence listing filed with the application follows.

SEQUENCE LISTING (7 sequences)

SEQ ID NO: 1 - DNA, 65 bp, Artificial Sequence
  Antisense nucleic acid against YB-1
actggggccggctgcggcagctgcgaaaaaaaaaaaaaaaaaaaaaaaaaaaaaaaaaaaaaaaa

SEQ ID NO: 2 - DNA, 65 bp, Artificial Sequence
  Sense strand of siRNA against c-Myc
agggauuccugggaaaacuggacggaaaaaaaaaaaaaaaaaaaaaaaaaaaaaaaaaaaaaaaa

SEQ ID NO: 3 - DNA, 25 bp, Artificial Sequence
  Antisense strand of siRNA against c-Myc
guccaguuuucccaggaaucccutt

SEQ ID NO: 4 - DNA, 64 bp, Artificial Sequence
  Sense strand of miRNA against KRAS
ugaggugcagugcugcaucucuggaaaaaaaaaaaaaaaaaaaaaaaaaaaaaaaaaaaaaaaa

SEQ ID NO: 5 - DNA, 24 bp, Artificial Sequence
  Antisense strand of miRNA against KRAS
ugagaugaagcacuguagcucatt

SEQ ID NO: 6 - DNA, 65 bp, Artificial Sequence
  Antisense nucleic acid against K-ras
cgggagtactggccgagccgccgccaaaaaaaaaaaaaaaaaaaaaaaaaaaaaaaaaaaaaaaa

SEQ ID NO: 7 - DNA, 60 bp, Artificial Sequence
  K3-dA40
atcgactctcgagcgttctcaaaaaaaaaaaaaaaaaaaaaaaaaaaaaaaaaaaaaaaa